European Patent Application EP 4 588 941 A1, published July 23, 2025. Title: NKG2D-NKP46 CELL ADAPTER MOLECULE AND USE THEREOF. Applicant: WEST CHINA HOSPITAL, SICHUAN UNIVERSITY. The sequence listing filed with the application follows.

SEQUENCE LISTING (18 sequences)

SEQ ID NO: 1 - protein, 139 aa, Homo sapiens
FLNSLFNQEVQIPLTESYCGPCPKNWICYKNNCYQFFDESKNWYESQASCMSQNASLLKVYSKEDQDLLKLVKSYHWMGLVHIPTNGSWQWEDGSILSPNLLTIIEMQKGDCALYASSFKGYIENCSTPNTYICMQRTV

SEQ ID NO: 2 - protein, 446 aa, synthetic construct
  source 1..446: note = anti-NKp46 Fab
QVQLVQSGAEVKKPGSSVKVSCKASGYTFSDYVINWVRQAPGQGLEWMGEIYPGSGTNYYNEKFKAKATITADKSTSTAYMELSSLRSEDTAVYYCARRGRYGLYAMDYWGQGTTVTVSSASTKGPSVFPLAPSSKSTSGGTAALGCLVKDYFPEPVTVSWNSGALTSGVHTFPAVLQSSGLYSLSSVVTVPSSSLGTQTYICNVNHKPSNTKVDKRVEPGGGGSGGGGSGGGGSDIQMTQSPSSLSASVGDRVTITCRASQDISNYLNWYQQKPGKAPKLLIYYTSRLHSGVPSRFSGSGSGTDFTFTISSLQPEDIATYFCQQGNTRPWTFGGGTKVEIKRTVAAPSVFIFPPSDEQLKSGTASVVCLLNNFYPREAKVQWKVDNALQSGNSQESVTEQDSKDSTYSLSSTLTLSKADYEKHKVYACEVTHQGLSSPVTKSFNR

SEQ ID NO: 3 - protein, 8 aa, synthetic construct
  source 1..8: note = anti-NKp46 HCDR1
GYTFSDYV

SEQ ID NO: 4 - protein, 8 aa, synthetic construct
  source 1..8: note = anti-NKp46 HCDR2
IYPGSGTN

SEQ ID NO: 5 - protein, 13 aa, synthetic construct
  source 1..13: note = anti-NKp46 HCDR3
ARRGRYGLYAMDY

SEQ ID NO: 6 - protein, 6 aa, synthetic construct
  source 1..6: note = anti-NKp46 LCDR1
QDISNY

SEQ ID NO: 7 - protein, 9 aa, synthetic construct
  source 1..9: note = anti-NKp46 LCDR3
QQGNTRPWT

SEQ ID NO: 8 - protein, 120 aa, synthetic construct
  source 1..120: note = anti-NKp46 VH
QVQLVQSGAEVKKPGSSVKVSCKASGYTFSDYVINWVRQAPGQGLEWMGEIYPGSGTNYYNEKFKAKATITADKSTSTAYMELSSLRSEDTAVYYCARRGRYGLYAMDYWGQGTTVTVSS

SEQ ID NO: 9 - protein, 108 aa, synthetic construct
  source 1..108: note = anti-NKp46 VL
DIQMTQSPSSLSASVGDRVTITCRASQDISNYLNWYQQKPGKAPKLLIYYTSRLHSGVPSRFSGSGSGTDFTFTISSLQPEDIATYFCQQGNTRPWTFGGGTKVEIKR

SEQ ID NO: 10 - protein, 243 aa, synthetic construct
  source 1..243: note = anti-NKp46 scFv
QVQLVQSGAEVKKPGSSVKVSCKASGYTFSDYVINWVRQAPGQGLEWMGEIYPGSGTNYYNEKFKAKATITADKSTSTAYMELSSLRSEDTAVYYCARRGRYGLYAMDYWGQGTTVTVSSGGGGSGGGGSGGGGSDIQMTQSPSSLSASVGDRVTITCRASQDISNYLNWYQQKPGKAPKLLIYYTSRLHSGVPSRFSGSGSGTDFTFTISSLQPEDIATYFCQQGNTRPWTFGGGTKVEIKR

SEQ ID NO: 11 - protein, 122 aa, synthetic construct
  source 1..122: note = anti-NKp46 VHH
QVQLVQSGAEVKKPGSSVKVSCKASGYTFSDYVINWVRQAPGQGLEWMGEIYPGSGTNYYNEKFKAKATITADKSTSTAYMELSSLRSEDTAVYYCARRGRYGLYAMDYWGQGTTVTVSSAS

SEQ ID NO: 12 - protein, 8 aa, synthetic construct
  source 1..8: note = anti-CD16 VHH CDR1
TLTFTPYR

SEQ ID NO: 13 - protein, 9 aa, synthetic construct
  source 1..9: note = anti-CD16 VHH CDR2
ISSGDGRTT

SEQ ID NO: 14 - protein, 12 aa, synthetic construct
  source 1..12: note = anti-CD16 VHH CDR3
NTFVSFVGIARS

SEQ ID NO: 15 - protein, 120 aa, synthetic construct
  source 1..120: note = anti-CD16 VHH
EVQLVESGGGFVQAGESLTLSCTSSTLTFTPYRMAWYRQAPGKQRDLVADISSGDGRTTNYADFAKGRFTISRDNIKNTVFLRMTNLKPEDTAVYYCNTFVSFVGIARSWGQGTQVTVSS

SEQ ID NO: 16 - protein, 231 aa, synthetic construct
  source 1..231: note = IgG Fc
PKSCDKTHTCPPCPAPELVGGPSVFLLPPKPKDTLMISRTPEVTCVVVDVSHEDPEVKFNWYVDGVEVHNAKTKPPEEQYNSTLRVVSVLTVLHQDWLNGKEYKCKVSNKALPAPIEKTISKAKGQPREPQVYTLPPSRDELTKNQVSLTCLVKGFYPSDIAVEWESNGQPENNYKTTPLVLDSDGSFFLYSKLTVDKSRWQQGNVFSCSVMHEALHNHYTQKSLSLSPGK

SEQ ID NO: 17 - protein, 114 aa, Homo sapiens
  source 1..114: note = IL-15
NWVNVISDLKKIEDLIQSMHIDATLYTESDVHPSCKVTAMKCFLLELQVISLESGDASIHDTVENLIILANNSLSSNGNVTESGCKECEELEEKNIKEFLQSFVHIVQMFINTS

SEQ ID NO: 18 - protein, 507 aa, synthetic construct
  source 1..507: note = Scfc (CH2-CH3-CH2-CH3)
APELLGGPSVFLFPPKPKDTLMTSRTPEVTCVVVDVSHEDPEVKFNWYVDGVEVHNAKTKPCEEQYNSTYRCVSVLTVLHQDWLNGKEYKCKVSNKALPAPIEKTISKAKGQPREPQVYTLPPSREEMTKNQVSLTCLVKGFYPSDIAVEWESNGQPENNYKTTPPVLDSDGSFFLYSKLTVDKSRWQQGNVFSCSVMHEALHNHYTQKSLSLSPGKGGGGSGGGGSGGGGSGGGGSGGGGSGGGGSGGGGSGGGGSGGGGSGGGGSGGGGSGGGGSGGGGSDKTHTCPPCPAPELLGGPSVFLFPPKPKDTLMTSRTPEVTCVVVDVSHEDPEVKFNWYVDGVEVHNAKTKPCEEQYNSTYRCVSVLTVLHQDWLNGKEYKCKVSNKALPAPIEKTISKAKGQPREPQVYTLPPSREEMTKNQVSLTCLVKGFYPSDIAVEWESNGQPENNYKTTPPVLDSDGSFFLYSKLTVDKSRWQQGNVFSCSVMHEALHNHYTQKSLSLSP